European Patent Application EP 4 198 131 A1, published June 21, 2023. Title: MICROORGANISMS FOR PRODUCING PUTRESCINE AND PROCESS FOR PRODUCING PUTRESCINE USING THEM. Applicant: CJ CheilJedang Corporation. The sequence listing filed with the application follows.

SEQUENCE LISTING (30 sequences)

SEQ ID NO: 1 - protein, 335 aa, Unknown
  C. glutamicum GNAT family N-acetyltransferase
MTPSLPRFRSQKPAVGDRVVARRRIPGANVHWTDAIGHVIGVDPLVVRPQSVGGMPSDAEEIVIPDDQLEVIKILSPRTIRNSDIRAVEVATAKAFPGLVNEWHDGWLLRAGDGIAERSNSASPLGPSVGFEPVPMEDISRFYARHDLPVKLHIPERIGRPAQKVIDADPQKWVMGPEILVMTKSLDHVESHELPGGLEFSVDKQPDQEWLGMYHFRGQALPAHALELLRTQIEGRMGFGRLTTPAGQTVAITRATITAAEERIFLGYSAVEVDPAFRRQGLGTALGSRIQEWGAEQHAQEAYLQVVAHNEAGIGLYQKLGFSEHHRHRYAERKF

SEQ ID NO: 2 - DNA, 1008 bp, Unknown
  C. glutamicum GNAT family N-acetyltransferase(Ncgl2644)
atgacgcctagtcttccccgtttccgcagccagaaacctgccgtcggcgatcgtgttgttgcacgtcgccggattcctggtgccaatgtgcattggacagatgccattggccatgtgattggggtggatccgttggtggttcgcccgcagtcggttggtgggatgccgtcggatgcggaagaaattgtcattcctgatgatcagcttgaggtgattaagattttgtcgccgcgcaccattaggaattcggatattcgtgcggtggaggttgccacggcgaaggcctttccggggctggtcaatgagtggcatgatggttggctgctgcgtgccggtgatggcattgcggagcgttctaattctgcgtcgccactcggcccaagtgttggttttgagccggtaccgatggaggatatttcgcggttttacgcaaggcacgatctccccgtgaagctgcacattccggagcggattggtcggcctgcgcagaaagtcattgacgccgatccccagaaatgggtgatgggcccggagattttggtgatgacgaaatctttggaccatgtggagtcgcacgagttgcccggtggcctagaatttagcgtcgataagcagcctgaccaggagtggctgggcatgtaccatttccgcggacaggcgttgcccgctcacgcccttgagcttttgcgcacgcaaatcgagggccgcatggggttcgggcgcctgaccacgccggcggggcaaaccgtcgcgatcacgcgcgccaccatcacggctgcggaggagcgcatatttttgggctattcagcggtcgaggtggatcctgcttttcgacgtcaggggctgggcaccgcgctcggctcgcgcatccaggagtggggcgccgagcaacacgcacaagaggcatatctccaggttgtcgcccataatgaagcaggtatcggcctgtatcaaaagctcgggttcagtgaacaccaccgacaccggtacgccgaacggaaattctaa

SEQ ID NO: 3 - protein, 408 aa, Unknown
  E.coli argE
MDKLLERFLNYVSLDTQSKAGVRQVPSTEGQWKLLHLLKEQLEEMGLINVTLSEKGTLMATLPANVPGDIPAIGFISHVDTSPDCSGKNVNPQIVENYRGGDIALGIGDEVLSPVMFPVLHQLLGQTLITTDGKTLLGADDKAGIAEIMTALAVLQQKKIPHGDIRVAFTPDEEVGKGAKHFDVDAFDARWAYTVDGGGVGELEFENFNAASVNIKIVGNNVHPGTAKGVMVNALSLAARIHAEVPADESPEMTEGYEGFYHLASMKGTVERADMHYIIRDFDRKQFEARKRKMMEIAKKVGKGLHPDCYIELVIEDSYYNMREKVVEHPHILDIAQQAMRDCDIEPELKPIRGGTDGAQLSFMGLPCPNLFTGGYNYHGKHEFVTLEGMEKAVQVIVRIAELTAQRK

SEQ ID NO: 4 - DNA, 1227 bp, Unknown
  E.coli argE
atggataaactacttgagcgatttttgaactacgtgtctctggatacccaatcaaaagcaggggtgagacaggttcccagcacggaaggccaatggaagttattgcatctgctgaaagagcagctcgaagagatggggcttatcaatgtgaccttaagtgagaagggcactttgatggcgacgttaccggctaacgtccctggcgatatcccggcgattggctttatttctcatgtggatacctcaccggattgcagcggcaaaaatgtgaatccgcaaattgttgaaaactatcgcggtggcgatattgcgctgggtatcggcgatgaagttttatcaccggttatgttcccggtgctgcatcagctactgggtcagacgctgattaccaccgatggtaaaaccttgttaggtgccgatgacaaagcaggtattgcagaaatcatgaccgcgctggcggtattgcaacagaaaaaaattccgcatggtgatattcgcgtcgcctttaccccggatgaagaagtgggcaaaggggcgaaacattttgatgttgacgccttcgatgcccgctgggcttacactgttgatggtggtggcgtaggcgaactggagtttgaaaacttcaacgccgcgtcggtcaatatcaaaattgtcggtaacaatgttcatccgggcacggcgaaaggagtgatggtaaatgcgctgtcgctggcggcacgtattcatgcggaagttccggcggatgaaagcccggaaatgacagaaggctatgaaggtttctatcatctggcgagcatgaaaggcaccgttgaacgggccgatatgcactacatcatccgtgatttcgaccgtaaacagtttgaagcgcgtaaacgtaaaatgatggagatcgccaaaaaagtgggcaaagggttacatcctgattgctacattgaactggtgattgaagacagttactacaatatgcgcgagaaagtggttgagcatccgcatattctcgatatcgcccagcaggcgatgcgcgattgcgatattgaaccggaactgaaaccgatccgcggtggtaccgacggcgcgcagttgtcgtttatgggattaccgtgcccgaacctgttcactggcggttacaactatcatggtaagcatgagtttgtgactctggaaggtatggaaaaagcggtgcaggtgatcgtccgtattgccgagttaacggcgcaacggaagtaa

SEQ ID NO: 5 - protein, 388 aa, Unknown
  C. glutamicum 13869 argJ
MAKKGITAPKGFVASATTAGIKASGNPDMALVVNQGPEFSAAAVFTRNRVFAAPVKVSRENVADGQIRAVLYNAGNANACNGLQGEKDARESVSHLAQNLGLEDSDIGVCSTGLIGELLPMDKLNTGIDQLTAEGALGDNGAAAAKAIMTTDTVDKETVVFADGWTVGGMGKGVGMMAPSLATMLVCLTTDASVTQEMAQIALANATAVTFDTLDIDGSTSTNDTVFLLASGASGITPTQDELNDAVYAACSDIAAKLQADAEGVTKRVAVTVVGTTNNEQAINAARTVARDNLFKCAMFGSDPNWGRVLAAVGMADADMEPEKISVFFNDQAVCLDSTGAPGAREVDLSGADIDVRIDLGTSGEGQATVRTTDLSFSYVEINSAYSS

SEQ ID NO: 6 - DNA, 1167 bp, Unknown
  C. glutamicum 13869 argJ
atggccaaaaaaggcattaccgcgccgaaaggcttcgttgcttctgcaacgaccgcgggtattaaagcttctggcaatcctgacatggcgttggtggttaaccagggtccagagttttccgcagcggccgtgtttacacgcaaccgagttttcgcagcgcctgtgaaggtgagccgggagaacgttgctgatggccagatcagggctgttttgtacaacgctggtaatgctaatgcgtgtaatggtctgcagggtgagaaggatgctcgtgagtctgtttctcatctagctcaaaatttgggcttggaggattccgatattggtgtgtgttccactggtcttattggtgagttgcttccgatggataagctcaatacaggtattgatcagctgaccgctgagggcgctttgggtgacaatggtgcagctgctgccaaggcgatcatgaccactgacacggtggataaggaaaccgtcgtgtttgctgatggttggactgtcggcggaatgggcaagggcgtgggcatgatggcgccgtctcttgccaccatgctggtctgcttgaccactgatgcatccgttactcaggaaatggctcagattgcgctggctaatgctacggccgttacgtttgacaccctggatattgatggatcaacctccaccaatgacaccgtgttcctgctggcatctggcgctagcggaatcaccccaactcaggatgaactcaacgatgcggtgtacgcagcttgttctgatatcgcagcgaagcttcaggctgatgcagagggggtgaccaagcgcgttgctgtgacagtggtgggaaccaccaacaacgagcaggcgatcaatgcggctcgcacggttgctcgtgacaatttgttcaagtgcgcaatgtttggatctgatccaaactggggtcgcgtgttggctgcagtcggcatggctgatgctgatatggaaccagagaagatttctgtgttcttcaatgatcaagcagtatgccttgattccactggcgctcctggtgctcgtgaggtggatctttccggcgctgacattgatgtccgaattgatttgggcaccagtggggaaggccaggcaacagttcgaaccactgacctgagcttctcctacgtggagatcaactccgcgtacagctcttaa

SEQ ID NO: 7 - protein, 388 aa, Unknown
  C. glutamicum 13032 argJ
MAEKGITAPKGFVASATTAGIKASGNPDMALVVNQGPEFSAAAVFTRNRVFAAPVKVSRENVADGQIRAVLYNAGNANACNGLQGEKDARESVSHLAQNLGLEDSDIGVCSTGLIGELLPMDKLNAGIDQLTAEGALGDNGAAAAKAIMTTDTVDKETVVFADGWTVGGMGKGVGMMAPSLATMLVCLTTDASVTQEMAQIALANATAVTFDTLDIDGSTSTNDTVFLLASGASGITPTQDELNDAVYAACSDIAAKLQADAEGVTKRVAVTVVGTTNNEQAINAARTVARDNLFKCAMFGSDPNWGRVLAAVGMADADMEPEKISVFFNGQAVCLDSTGAPGAREVDLSGADIDVRIDLGTSGEGQATVRTTDLSFSYVEINSAYSS

SEQ ID NO: 8 - DNA, 1167 bp, Unknown
  C. glutamicum 13032 argJ
atggcagaaaaaggcattaccgcgccgaaaggcttcgttgcttctgcaacgaccgcgggtattaaagcttctggcaatcctgacatggcgttggtggttaaccagggtccagagttttccgcagcggccgtgtttacacgtaaccgagttttcgcagcgcctgtgaaggtgagccgagagaacgttgctgatggccagatcagggctgttttgtacaacgctggtaatgctaatgcgtgtaatggtctgcagggtgagaaggatgctcgtgagtctgtttctcatctagctcaaaatttgggcttggaggattccgatattggtgtgtgttccactggtcttattggtgagttgcttccgatggataagctcaatgcaggtattgatcagctgaccgctgagggcgctttgggtgacaatggtgcagctgctgccaaggcgatcatgaccactgacacggtggataaggaaaccgtcgtgtttgctgatggttggactgtcggcggaatgggcaagggcgtgggcatgatggcgccgtctcttgccaccatgctggtctgcttgaccactgatgcatccgttactcaggaaatggctcagatcgcgctggctaatgctacggccgttacgtttgacaccctggatattgatggatcaacctccaccaatgacaccgtgttcctgctggcatctggcgctagcggaatcaccccaactcaggatgaactcaacgatgcggtgtacgcagcttgttctgatatcgcagcgaagcttcaggctgatgcagagggtgtgaccaagcgcgttgctgtgacagtggtgggaaccaccaacaacgagcaggcgattaatgcggctcgcactgttgctcgtgacaatttgttcaagtgcgcaatgtttggatctgatccaaactggggtcgcgtgttggctgcagtcggcatggctgatgctgatatggaaccagagaagatttctgtgttcttcaatggtcaagcagtatgccttgattccactggcgctcctggtgctcgtgaggtggatctttccggcgctgacattgatgtccgaattgatttgggcaccagtggggaaggccaggcaacagttcgaaccactgacctgagcttctcctacgtggagatcaactccgcgtacagctcttaa

SEQ ID NO: 9 - DNA, 289 bp, Unknown
  lysCP1
ccgatgctagggcgaaaagcacggcgagcagattgctttgcacttgattcagggtagttgactaaagagttgctcgcgaagtagcacctgtcacttttgtctcaaatattaaatcgaatatcaatatatggtctgtttattggaacgcgtcccagtggctgagacgcatccgctaaagccccaggaaccctgtgcagaaagaaaacactcctctggctaggtagacacagtttattgtggtagagttgagcgggtaactgtcagcacgtagatcgaaaggtgcacaaag

SEQ ID NO: 10 - DNA, 36 bp, Artificial Sequence
  Tn-A-F
atcctctagagtcgaccatcgctgacaccatctgcc

SEQ ID NO: 11 - DNA, 38 bp, Artificial Sequence
  Tn-A-R
gggcccactagtctcgagttcaccgcgggagccaagcc

SEQ ID NO: 12 - DNA, 37 bp, Artificial Sequence
  Tn-B-F
ctcgagactagtgggccctggattccaaggctacgcc

SEQ ID NO: 13 - DNA, 36 bp, Artificial Sequence
  Tn-B-R
atgcctgcaggtcgaccctgaatggataaggcaccg

SEQ ID NO: 14 - DNA, 510 bp, Unknown
  Tn-A
gcagacgcactcgactacacctccacctgcccagaatgctcccaacctggggtgtttcgtcatcacacccaccggatgctcattgatttacccatcgtcgggtttcccaccaaactgtttatccgtctacctcgctaccgctgcaccaaccccacatgtaagcaaaagtatttccaagcagaactaagctgcgctgaccacggtaaaaaggtcacccaccgggtcacccgctggattttacaacgccttgctattgaccggatgagtgttcacgcaaccgcgaaagcacttgggctagggtgggatttaacctgccaactagccctcgatatgtgccgtgagctggtctataacgatcctcaccatcttgatggagtgtatgtcattggggtggatgagcataagtggtcacataatagggctaagcatggtgatgggtttgtcaccgtgattgtcgatatgaccgggcatcggtatgactcacggtgtcctgcccggttattagatgtc

SEQ ID NO: 15 - DNA, 479 bp, Unknown
  Tn-B
aactcattccttctgctcgtcgcgtgatggatccattccatgttgtgcggcttgctggtgacaagctcaccgcctgccggcaacgcctccagcgggagaaataccagcgtcgtggtttaagccaggatccgttgtataaaaaccggaagaccttgttgaccacgcacaagtggttgagtcctcgtcagcaagaaagcttggagcagttgtgggcgtatgacaaagactacggggcgttaaagcttgcgtggcttgcgtatcaggcgattattgattgttatcagatgggtaataagcgtgaagcgaagaagaaaatgcggaccattattgatcagcttcgggtgttgaaggggccgaataaggaactcgcgcagttgggtcgtagtttgtttaaacgacttggtgatgtgttggcgtatttcgatgttggtgtctccaacggtccggtcgaagcgatcaacggacggttggagcatttg

SEQ ID NO: 16 - DNA, 34 bp, Artificial Sequence
  lysCP1 promotor_F
gaatgagttcctcgagccgatgctagggcgaaaa

SEQ ID NO: 17 - DNA, 36 bp, Artificial Sequence
  lysCP1 promotor_R
ctttgtgcacctttcgatctacgtgctgacagttac

SEQ ID NO: 18 - DNA, 27 bp, Artificial Sequence
  argJ _F
gttccacatggccaaaaaaggcattac

SEQ ID NO: 19 - DNA, 34 bp, Artificial Sequence
  argJ _R
ttctttttaagagctgtacgcggagttgatctcc

SEQ ID NO: 20 - DNA, 1332 bp, Unknown
  E.coli arg A
gtggtaaaggaacgtaaaaccgagttggtcgagggattccgccattcggttccctatatcaatacccaccggggaaaaacgtttgtcatcatgctcggcggtgaagccattgagcatgagaatttctccagtatcgttaatgatatcgggttgttgcacagcctcggcatccgtctggtggtggtctatggcgcacgtccgcagatcgacgcaaatctggctgcgcatcaccacgaaccgctgtatcacaagaatatacgtgtgaccgacgccaaaacactggaactggtgaagcaggctgcgggaacattgcaactggatattactgctcgcctgtcgatgagtctcaataacacgccgctgcagggcgcgcatatcaacgtcgtcagtggcaattttattattgcccagccgctgggcgtcgatgacggcgtggattactgccatagcgggcgtatccggcggattgatgaagacgcgatccatcgtcaactggacagcggtgcaatagtgctaatggggccggtcgctgtttcagtcactggcgagagctttaacctgacctcggaagagattgccactcaactggccatcaaactgaaagctgaaaagatgattggtttttgctcttcccagggcgtcactaatgacgacggtgatattgtctccgaacttttccctaacgaagcgcaagcgcgggtagaagcccaggaagagaaaggcgattacaactccggtacggtgcgctttttgcgtggcgcagtgaaagcctgccgcagcggcgtgcgtcgctgtcatttaatcagttatcaggaagatggcgcgctgttgcaagagttgttctcacgcgacggtatcggtacgcagattgtgatggaaagcgccgagcagattcgtcgcgcaacaatcaacgatattggcggtattctggagttgattcgcccactggagcagcaaggtattctggtacgccgttctcgcgagcagctggagatggaaatcgacaaattcaccattattcagcgcgataacacgactattgcctgcgccgcgctctatccgttcccggaagagaagattggggaaatggcctgtgtggcagttcacccggattaccgcagttcatcaaggggtgaagttctgctggaacgcattgccgctcaggcgaagcagagcggcttaagcaaattgtttgtgctgaccacgcgcagtattcactggttccaggaacgtggatttaccccagtggatattgatttactgcccgagagcaaaaagcagttgtacaactaccagcgtaaatccaaagtgttgatggcggatttagggtaa

SEQ ID NO: 21 - DNA, 37 bp, Artificial Sequence
  argA ORF_F
gaaaggtgcacaaagatggtaaaggaacgtaaaaccg

SEQ ID NO: 22 - DNA, 34 bp, Artificial Sequence
  argA ORF_R
gcccactagtctcgagcatgcggcgttgattttg

SEQ ID NO: 23 - DNA, 35 bp, Artificial Sequence
  argE ORF_F
gaaaggtgcacaaagatgaaaaacaaattaccgcc

SEQ ID NO: 24 - DNA, 36 bp, Artificial Sequence
  argE ORF_R
gcccactagtctcgaggtttgagtcactgtcggtcg

SEQ ID NO: 25 - DNA, 38 bp, Artificial Sequence
  Ncgl2644 ORF_F
gaggagatcaaaacacatatgacgcctagtcttccccg

SEQ ID NO: 26 - DNA, 23 bp, Artificial Sequence
  Ncgl2644 ORF_R
ttagaatttccgttcggcgtacc

SEQ ID NO: 27 - DNA, 25 bp, Artificial Sequence
  argJ_N_F
cgggatcccacgcctgtctggtcgc

SEQ ID NO: 28 - DNA, 29 bp, Artificial Sequence
  argJ_N_R
acgcgtcgacggatctaaagcggcgcttc

SEQ ID NO: 29 - DNA, 32 bp, Artificial Sequence
  argJ_C_F
acgcgtcgactccggcgctgacattgatgtcc

SEQ ID NO: 30 - DNA, 29 bp, Artificial Sequence
  argJ_C_R
ctagtctagagagctgcaccaggtagacg